European Patent Application EP 4 748 931 A1, published May 27, 2026. Title: DON 분해 활성을 갖는 신규 폴리펩티드. Applicant: 씨제이제일제당 주식회사. The sequence listing filed with the application follows.

SEQUENCE LISTING (74 sequences)

SEQ ID NO: 1 - protein, 182 aa, synthetic construct
MASSGPKESAANNPGLQTPPDEATKGYFMQQTMFRIKDPKVSLDFYSRVLGMSLLKRIDVPDMKMTLYFMGYEDVSSAPSDPIERTAWTFGRPATIELTHKWGTESDPEFKGYHNGNSEPIGFGHIGITVDDTYKACERFERLGVEFVKKPDDGYAFIKDPDGYWIEIFDLKNIRNVVNGVA

SEQ ID NO: 2 - DNA, 546 bp, synthetic construct
  source 1..546: mol_type = other DNA
atggcatcgtccgggccgaaagagtcggctgccaataatcctggcttgcaaactccacctgacgaggccactaagggttattttatgcaacagacaatgtttcgcattaaagaccctaaagtgtctttggacttctattcgcgcgtgcttggtatgagccttttgaaaagaattgacgtcccggatatgaagatgacgttatattttatgggatatgaagatgtaagtagtgcgccaagtgatccaatagagcggaccgcctggacatttggcagaccagcgacaatcgaattgacccataagtggggtaccgagagcgacccggagtttaaaggttaccataatggcaattctgaaccaattggtttcgggcacataggcatcacggtcgatgacacttacaaggcgtgtgagagattcgaacgtcttggggtagaatttgtgaaaaagccggatgacggctatgcgtttattaaagaccccgatggctactggatagagatatttgacttgaagaatatacgcaatgtggtaaatggagtcgct

SEQ ID NO: 3 - protein, 182 aa, synthetic construct
MASSGPKESAANNPGLQTPPDEATKGYIMQQTMFRIKDPKVSLDFYSRVLGMSLLKRIDVPDMKMTLYFMGYEDVSSAPSDPIERTAWTFGRPATIELTHKWGTESDPEFKGYHNGNSEPIGFGHIGITVDDTYKACERFERLGVEFVKKPDDGYAFIKDPDGYWIEIFDLKNIRNVVNGVA

SEQ ID NO: 4 - DNA, 546 bp, synthetic construct
  source 1..546: mol_type = other DNA
atggcatcgtccgggccgaaagagtcggctgccaataatcctggcttgcaaactccacctgacgaggccactaagggttatattatgcaacagacaatgtttcgcattaaagaccctaaagtgtctttggacttctattcgcgcgtgcttggtatgagccttttgaaaagaattgacgtcccggatatgaagatgacgttatattttatgggatatgaagatgtaagtagtgcgccaagtgatccaatagagcggaccgcctggacatttggcagaccagcgacaatcgaattgacccataaatggggtaccgagagcgacccggagtttaaaggttaccataatggcaattctgaaccaattggtttcgggcacataggcatcacggtcgatgacacttacaaggcgtgtgagagattcgaacgtcttggggtagaatttgtgaaaaagccggatgacggctatgcgtttattaaagaccccgatggctactggatagagatatttgacttgaagaatatacgcaatgtggtaaatggagtcgct

SEQ ID NO: 5 - protein, 182 aa, synthetic construct
MASSGPKESAANNPGLQTPPDEATKGYFMQQTMFRIKDPKVSLDFYSRVLGMSLLKRIDVPDMKMTLYFMGYEDVSSAPSDPIERTAWTFGRPATIELTHFWGTESDPEFKGYHNGNSEPIGFGHIGITVDDTYKACERFERLGVEFVKKPDDGYAFIKDPDGYWIEIFDLKNIRNVVNGVA

SEQ ID NO: 6 - DNA, 546 bp, synthetic construct
  source 1..546: mol_type = other DNA
atggcatcgtccgggccgaaagagtcggctgccaataatcctggcttgcaaactccacctgacgaggccactaagggttattttatgcaacagacaatgtttcgcattaaagaccctaaagtgtctttggacttctattcgcgcgtgcttggtatgagccttttgaaaagaattgacgtcccggatatgaagatgacgttatattttatgggatatgaagatgtaagtagtgcgccaagtgatccaatagagcggaccgcctggacatttggcagaccagcgacaatcgaattgacccatttttggggtaccgagagcgacccggagtttaaaggttaccataatggcaattctgaaccaattggtttcgggcacataggcatcacggtcgatgacacttacaaggcgtgtgagagattcgaacgtcttggggtagaatttgtgaaaaagccggatgacggctatgcgtttattaaagaccccgatggctactggatagagatatttgacttgaagaatatacgcaatgtggtaaatggagtcgct

SEQ ID NO: 7 - protein, 182 aa, synthetic construct
MASSGPKESAANNPGLQTPPDEATKGYFMQQTMFRIKDPKVSLDFYSRVLGMSLLKRIDVPDMKMTLYFMGYEDVSSAPSDPIERTAWTFGRPATIELTHKWGTESDPEFKGYHNGNSEPIGFGHIGITVDDTYKACERFERLGVEFVKKPGDGYAFIKDPDGYWIEIFDLKNIRNVVNGVA

SEQ ID NO: 8 - DNA, 546 bp, synthetic construct
  source 1..546: mol_type = other DNA
atggcatcgtccgggccgaaagagtcggctgccaataatcctggcttgcaaactccacctgacgaggccactaagggttattttatgcaacagacaatgtttcgcattaaagaccctaaagtgtctttggacttctattcgcgcgtgcttggtatgagccttttgaaaagaattgacgtcccggatatgaagatgacgttatattttatgggatatgaagatgtaagtagtgcgccaagtgatccaatagagcggaccgcctggacatttggcagaccagcgacaatcgaattgacccataagtggggtaccgagagcgacccggagtttaaaggttaccataatggcaattctgaaccaattggtttcgggcacataggcatcacggtcgatgacacttacaaggcgtgtgagagattcgaacgtcttggggtagaatttgtgaaaaagccgggcgacggctatgcgtttattaaagaccccgatggctactggatagagatatttgacttgaagaatatacgcaatgtggtaaatggagtcgct

SEQ ID NO: 9 - protein, 182 aa, synthetic construct
MASSGPKESAANNPGLQTPPDEATKGYIMQQTMFRIKDPKVSLDFYSRVLGMSLLKRIDVPDMKMTLYFMGYEDVSSAPSDPIERTAWTFGRPATIELTHFWGTESDPEFKGYHNGNSEPIGFGHIGITVDDTYKACERFERLGVEFVKKPDDGYAFIKDPDGYWIEIFDLKNIRNVVNGVA

SEQ ID NO: 10 - DNA, 546 bp, synthetic construct
  source 1..546: mol_type = other DNA
atggcatcgtccgggccgaaagagtcggctgccaataatcctggcttgcaaactccacctgacgaggccactaagggttatattatgcaacagacaatgtttcgcattaaagaccctaaagtgtctttggacttctattcgcgcgtgcttggtatgagccttttgaaaagaattgacgtcccggatatgaagatgacgttatattttatgggatatgaagatgtaagtagtgcgccaagtgatccaatagagcggaccgcctggacatttggcagaccagcgacaatcgaattgacccatttttggggtaccgagagcgacccggagtttaaaggttaccataatggcaattctgaaccaattggtttcgggcacataggcatcacggtcgatgacacttacaaggcgtgtgagagattcgaacgtcttggggtagaatttgtgaaaaagccggatgacggctatgcgtttattaaagaccccgatggctactggatagagatatttgacttgaagaatatacgcaatgtggtaaatggagtcgct

SEQ ID NO: 11 - protein, 182 aa, synthetic construct
MASSGPKESAANNPGLQTPPDEATKGYIMQQTMFRIKDPKVSLDFYSRVLGMSLLKRIDVPDMKMTLYFMGYEDVSSAPSDPIERTAWTFGRPATIELTHKWGTESDPEFKGYHNGNSEPIGFGHIGITVDDTYKACERFERLGVEFVKKPGDGYAFIKDPDGYWIEIFDLKNIRNVVNGVA

SEQ ID NO: 12 - DNA, 546 bp, synthetic construct
  source 1..546: mol_type = other DNA
atggcatcgtccgggccgaaagagtcggctgccaataatcctggcttgcaaactccacctgacgaggccactaagggttatattatgcaacagacaatgtttcgcattaaagaccctaaagtgtctttggacttctattcgcgcgtgcttggtatgagccttttgaaaagaattgacgtcccggatatgaagatgacgttatattttatgggatatgaagatgtaagtagtgcgccaagtgatccaatagagcggaccgcctggacatttggcagaccagcgacaatcgaattgacccataaatggggtaccgagagcgacccggagtttaaaggttaccataatggcaattctgaaccaattggtttcgggcacataggcatcacggtcgatgacacttacaaggcgtgtgagagattcgaacgtcttggggtagaatttgtgaaaaagccgggcgacggctatgcgtttattaaagaccccgatggctactggatagagatatttgacttgaagaatatacgcaatgtggtaaatggagtcgct

SEQ ID NO: 13 - protein, 182 aa, synthetic construct
MASSGPKESAANNPGLQTPPDEATKGYIMQQTMFRIKDPKVSLDFYSRVLGMSLLKRIDVPDMKMTLYFMGYEDVSSAPSDPIERTAWTFGRPATIELTHFWGTESDPEFKGYHNGNSEPIGFGHIGITVDDTYKACERFERLGVEFVKKPGDGYAFIKDPDGYWIEIFDLKNIRNVVNGVA

SEQ ID NO: 14 - DNA, 546 bp, synthetic construct
  source 1..546: mol_type = other DNA
atggcatcgtccgggccgaaagagtcggctgccaataatcctggcttgcaaactccacctgacgaggccactaagggttatattatgcaacagacaatgtttcgcattaaagaccctaaagtgtctttggacttctattcgcgcgtgcttggtatgagccttttgaaaagaattgacgtcccggatatgaagatgacgttatattttatgggatatgaagatgtaagtagtgcgccaagtgatccaatagagcggaccgcctggacatttggcagaccagcgacaatcgaattgacccatttttggggtaccgagagcgacccggagtttaaaggttaccataatggcaattctgaaccaattggtttcgggcacataggcatcacggtcgatgacacttacaaggcgtgtgagagattcgaacgtcttggggtagaatttgtgaaaaagccgggggacggctatgcgtttattaaagaccccgatggctactggatagagatatttgacttgaagaatatacgcaatgtggtaaatggagtcgct

SEQ ID NO: 15 - DNA, 42 bp, synthetic construct
  source 1..42: mol_type = other DNA
ggccactaagggttatattatgcaacagacaatgtttcgcat

SEQ ID NO: 16 - DNA, 43 bp, synthetic construct
  source 1..43: mol_type = other DNA
cataatataacccttagtggcctcgtcaggtggagtttgcaag

SEQ ID NO: 17 - DNA, 41 bp, synthetic construct
  source 1..41: mol_type = other DNA
atttttggggtaccgagagcgacccggagtttaaaggttac

SEQ ID NO: 18 - DNA, 39 bp, synthetic construct
  source 1..39: mol_type = other DNA
gctctcggtaccccaaaaatgggtcaattcgattgtcgc

SEQ ID NO: 19 - DNA, 48 bp, synthetic construct
  source 1..48: mol_type = other DNA
agaatttgtgaaaaagccgggcgacggctatgcgtttattaaagaccc

SEQ ID NO: 20 - DNA, 49 bp, synthetic construct
  source 1..49: mol_type = other DNA
gcccggctttttcacaaattctaccccaagacgttcgaatctctcacac

SEQ ID NO: 21 - protein, 182 aa, synthetic construct
MASSGPKESAANNPGLQTPPDEATKGYFMQQTMFRIKDPKVSLDFYSRVLGMSLLKRIDVPDMKFTLYFMGYEDVSSAPSDPIERTAWTFGRPATIELTHKWGTESDPEFKGYHNGNSEPRGFGHIGITVDDTYKACERFERLGVEFVKKPDDGYAFIKDPDGYWIEIFDLKNIRNVVNGVA

SEQ ID NO: 22 - DNA, 546 bp, synthetic construct
  source 1..546: mol_type = other DNA
atggcatcgtccgggccgaaagagtcggctgccaataatcctggcttgcaaactccacctgacgaggccactaagggttattttatgcaacagacaatgtttcgcattaaagaccctaaagtgtctttggacttctattcgcgcgtgcttggtatgagccttttgaaaagaattgacgtcccggatatgaagttcacgttatattttatgggatatgaagatgtaagtagtgcgccaagtgatccaatagagcggaccgcctggacatttggcagaccagcgacaatcgaattgacccataagtggggtaccgagagcgacccggagtttaaaggttaccataatggcaattctgaaccacggggtttcgggcacataggcatcacggtcgatgacacttacaaggcgtgtgagagattcgaacgtcttggggtagaatttgtgaaaaagccggatgacggctatgcgtttattaaagaccccgatggctactggatagagatatttgacttgaagaatatacgcaatgtggtaaatggagtcgct

SEQ ID NO: 23 - protein, 182 aa, synthetic construct
MGSLDSKESPANNPGLHSPPDEATKGYILQQTMFRIKDPKPALEFYSRVLGMSLLNKVDVPYMKMTLYMMGYEDVSSAPSDPVEKTIWTFGRPATMELTHFWGTENDPEFKGYHDGNSEPTGFGHIGITVDDMYKACERFESLGVEFVKKPGDGYAFIKDPDGYWIEIFDLNGIRAIVNNLA

SEQ ID NO: 24 - DNA, 546 bp, synthetic construct
  source 1..546: mol_type = other DNA
atggggtcccttgatagcaaagaatcgcccgctaataaccctggacttcatagtccccccgacgaggccacaaaaggctacatccttcaacaaactatgttccgcataaaagacccgaagccagcactggagttctattctagagtattggggatgtcattactgaacaaagtggatgtaccatacatgaaaatgaccctgtacatgatgggttacgaagatgtttcatctgccccaagcgatcccgtcgagaagactatttggacgttcggccgtcctgcaacgatggaactgacccatttttgggggaccgagaatgaccccgaatttaagggttaccatgacgggaactcagaacctaccggttttggccatattggtattactgtggatgatatgtataaagcgtgcgagcggtttgagagccttggtgttgaatttgttaaaaaaccaggagacggatatgcttttatcaaggacccggacggctactggattgagatttttgatttgaacggaatacgggctatcgtaaataacttagca

SEQ ID NO: 25 - DNA, 49 bp, synthetic construct
  source 1..49: mol_type = other DNA
ggccactaagggttattttctgcaacagacaatgtttcgcattaaagac

SEQ ID NO: 26 - DNA, 45 bp, synthetic construct
  source 1..45: mol_type = other DNA
cagaaaataacccttagtggcctcgtcaggtggagtttgcaagcc

SEQ ID NO: 27 - DNA, 38 bp, synthetic construct
  source 1..38: mol_type = other DNA
agcggaccatttggacatttggcagaccagcgacaatc

SEQ ID NO: 28 - DNA, 39 bp, synthetic construct
  source 1..39: mol_type = other DNA
aaatgtccaaatggtccgctctattggatcacttggcgc

SEQ ID NO: 29 - DNA, 39 bp, synthetic construct
  source 1..39: mol_type = other DNA
cctggacatttagcagaccagcgacaatcgaattgaccc

SEQ ID NO: 30 - DNA, 39 bp, synthetic construct
  source 1..39: mol_type = other DNA
tggtctgctaaatgtccaggcggtccgctctattggatc

SEQ ID NO: 31 - protein, 182 aa, synthetic construct
MASSGPKESAANNPGLQTPPDEATKGYFLQQTMFRIKDPKVSLDFYSRVLGMSLLKRIDVPDMKMTLYFMGYEDVSSAPSDPIERTAWTFGRPATIELTHKWGTESDPEFKGYHNGNSEPIGFGHIGITVDDTYKACERFERLGVEFVKKPDDGYAFIKDPDGYWIEIFDLKNIRNVVNGVA

SEQ ID NO: 32 - DNA, 546 bp, synthetic construct
  source 1..546: mol_type = other DNA
atggcatcgtccgggccgaaagagtcggctgccaataatcctggcttgcaaactccacctgacgaggccactaagggttattttctgcaacagacaatgtttcgcattaaagaccctaaagtgtctttggacttctattcgcgcgtgcttggtatgagccttttgaaaagaattgacgtcccggatatgaagatgacgttatattttatgggatatgaagatgtaagtagtgcgccaagtgatccaatagagcggaccgcctggacatttggcagaccagcgacaatcgaattgacccataagtggggtaccgagagcgacccggagtttaaaggttaccataatggcaattctgaaccaattggtttcgggcacataggcatcacggtcgatgacacttacaaggcgtgtgagagattcgaacgtcttggggtagaatttgtgaaaaagccggatgacggctatgcgtttattaaagaccccgatggctactggatagagatatttgacttgaagaatatacgcaatgtggtaaatggagtcgct

SEQ ID NO: 33 - protein, 182 aa, synthetic construct
MASSGPKESAANNPGLQTPPDEATKGYFMQQTMFRIKDPKVSLDFYSRVLGMSLLKRIDVPDMKMTLYFMGYEDVSSAPSDPIERTIWTFGRPATIELTHKWGTESDPEFKGYHNGNSEPIGFGHIGITVDDTYKACERFERLGVEFVKKPDDGYAFIKDPDGYWIEIFDLKNIRNVVNGVA

SEQ ID NO: 34 - DNA, 546 bp, synthetic construct
  source 1..546: mol_type = other DNA
atggcatcgtccgggccgaaagagtcggctgccaataatcctggcttgcaaactccacctgacgaggccactaagggttattttatgcaacagacaatgtttcgcattaaagaccctaaagtgtctttggacttctattcgcgcgtgcttggtatgagccttttgaaaagaattgacgtcccggatatgaagatgacgttatattttatgggatatgaagatgtaagtagtgcgccaagtgatccaatagagcggaccatttggacatttggcagaccagcgacaatcgaattgacccataagtggggtaccgagagcgacccggagtttaaaggttaccataatggcaattctgaaccaattggtttcgggcacataggcatcacggtcgatgacacttacaaggcgtgtgagagattcgaacgtcttggggtagaatttgtgaaaaagccggatgacggctatgcgtttattaaagaccccgatggctactggatagagatatttgacttgaagaatatacgcaatgtggtaaatggagtcgct

SEQ ID NO: 35 - protein, 182 aa, synthetic construct
MASSGPKESAANNPGLQTPPDEATKGYFMQQTMFRIKDPKVSLDFYSRVLGMSLLKRIDVPDMKMTLYFMGYEDVSSAPSDPIERTAWTFSRPATIELTHKWGTESDPEFKGYHNGNSEPIGFGHIGITVDDTYKACERFERLGVEFVKKPDDGYAFIKDPDGYWIEIFDLKNIRNVVNGVA

SEQ ID NO: 36 - DNA, 546 bp, synthetic construct
  source 1..546: mol_type = other DNA
atggcatcgtccgggccgaaagagtcggctgccaataatcctggcttgcaaactccacctgacgaggccactaagggttattttatgcaacagacaatgtttcgcattaaagaccctaaagtgtctttggacttctattcgcgcgtgcttggtatgagccttttgaaaagaattgacgtcccggatatgaagatgacgttatattttatgggatatgaagatgtaagtagtgcgccaagtgatccaatagagcggaccgcctggacatttagcagaccagcgacaatcgaattgacccataagtggggtaccgagagcgacccggagtttaaaggttaccataatggcaattctgaaccaattggtttcgggcacataggcatcacggtcgatgacacttacaaggcgtgtgagagattcgaacgtcttggggtagaatttgtgaaaaagccggatgacggctatgcgtttattaaagaccccgatggctactggatagagatatttgacttgaagaatatacgcaatgtggtaaatggagtcgct

SEQ ID NO: 37 - DNA, 51 bp, synthetic construct
  source 1..51: mol_type = other DNA
gtacaggaaagaactatatttttcgtggatgacgggaactacaagacacgt

SEQ ID NO: 38 - DNA, 30 bp, synthetic construct
  source 1..30: mol_type = other DNA
atccacgaaaaatatagttctttcctgtac

SEQ ID NO: 39 - DNA, 51 bp, synthetic construct
  source 1..51: mol_type = other DNA
gtacaggaaagaactatatttttcctggatgacgggaactacaagacacgt

SEQ ID NO: 40 - DNA, 30 bp, synthetic construct
  source 1..30: mol_type = other DNA
atccaggaaaaatatagttctttcctgtac

SEQ ID NO: 41 - DNA, 51 bp, synthetic construct
  source 1..51: mol_type = other DNA
gtacaggaaagaactatatttttcagcgatgacgggaactacaagacacgt

SEQ ID NO: 42 - DNA, 30 bp, synthetic construct
  source 1..30: mol_type = other DNA
atcgctgaaaaatatagttctttcctgtac

SEQ ID NO: 43 - DNA, 51 bp, synthetic construct
  source 1..51: mol_type = other DNA
gtacaggaaagaactatatttttcccggatgacgggaactacaagacacgt

SEQ ID NO: 44 - DNA, 30 bp, synthetic construct
  source 1..30: mol_type = other DNA
atccgggaaaaatatagttctttcctgtac

SEQ ID NO: 45 - DNA, 51 bp, synthetic construct
  source 1..51: mol_type = other DNA
gtacaggaaagaactatatttttcatggatgacgggaactacaagacacgt

SEQ ID NO: 46 - DNA, 30 bp, synthetic construct
  source 1..30: mol_type = other DNA
atccatgaaaaatatagttctttcctgtac

SEQ ID NO: 47 - DNA, 51 bp, synthetic construct
  source 1..51: mol_type = other DNA
gtacaggaaagaactatatttttcaacgatgacgggaactacaagacacgt

SEQ ID NO: 48 - DNA, 30 bp, synthetic construct
  source 1..30: mol_type = other DNA
atcgttgaaaaatatagttctttcctgtac

SEQ ID NO: 49 - DNA, 51 bp, synthetic construct
  source 1..51: mol_type = other DNA
gtacaggaaagaactatatttttcggcgatgacgggaactacaagacacgt

SEQ ID NO: 50 - DNA, 30 bp, synthetic construct
  source 1..30: mol_type = other DNA
atcgccgaaaaatatagttctttcctgtac

SEQ ID NO: 51 - DNA, 51 bp, synthetic construct
  source 1..51: mol_type = other DNA
gtacaggaaagaactatatttttcgaagatgacgggaactacaagacacgt

SEQ ID NO: 52 - DNA, 30 bp, synthetic construct
  source 1..30: mol_type = other DNA
atcttcgaaaaatatagttctttcctgtac

SEQ ID NO: 53 - DNA, 51 bp, synthetic construct
  source 1..51: mol_type = other DNA
gtacaggaaagaactatatttttcattgatgacgggaactacaagacacgt

SEQ ID NO: 54 - DNA, 30 bp, synthetic construct
  source 1..30: mol_type = other DNA
atcaatgaaaaatatagttctttcctgtac

SEQ ID NO: 55 - DNA, 51 bp, synthetic construct
  source 1..51: mol_type = other DNA
gtacaggaaagaactatatttttctgggatgacgggaactacaagacacgt

SEQ ID NO: 56 - DNA, 30 bp, synthetic construct
  source 1..30: mol_type = other DNA
atcccagaaaaatatagttctttcctgtac

SEQ ID NO: 57 - DNA, 51 bp, synthetic construct
  source 1..51: mol_type = other DNA
gtacaggaaagaactatatttttctttgatgacgggaactacaagacacgt

SEQ ID NO: 58 - DNA, 30 bp, synthetic construct
  source 1..30: mol_type = other DNA
atcaaagaaaaatatagttctttcctgtac

SEQ ID NO: 59 - DNA, 51 bp, synthetic construct
  source 1..51: mol_type = other DNA
gtacaggaaagaactatatttttccgtgatgacgggaactacaagacacgt

SEQ ID NO: 60 - DNA, 30 bp, synthetic construct
  source 1..30: mol_type = other DNA
atcacggaaaaatatagttctttcctgtac

SEQ ID NO: 61 - DNA, 51 bp, synthetic construct
  source 1..51: mol_type = other DNA
gtacaggaaagaactatatttttccatgatgacgggaactacaagacacgt

SEQ ID NO: 62 - DNA, 30 bp, synthetic construct
  source 1..30: mol_type = other DNA
atcatggaaaaatatagttctttcctgtac

SEQ ID NO: 63 - DNA, 51 bp, synthetic construct
  source 1..51: mol_type = other DNA
gtacaggaaagaactatatttttctatgatgacgggaactacaagacacgt

SEQ ID NO: 64 - DNA, 30 bp, synthetic construct
  source 1..30: mol_type = other DNA
atcatagaaaaatatagttctttcctgtac

SEQ ID NO: 65 - DNA, 51 bp, synthetic construct
  source 1..51: mol_type = other DNA
gtacaggaaagaactatatttttcgcggatgacgggaactacaagacacgt

SEQ ID NO: 66 - DNA, 30 bp, synthetic construct
  source 1..30: mol_type = other DNA
atccgcgaaaaatatagttctttcctgtac

SEQ ID NO: 67 - DNA, 51 bp, synthetic construct
  source 1..51: mol_type = other DNA
gtacaggaaagaactatatttttcaccgatgacgggaactacaagacacgt

SEQ ID NO: 68 - DNA, 30 bp, synthetic construct
  source 1..30: mol_type = other DNA
atcggtgaaaaatatagttctttcctgtac

SEQ ID NO: 69 - DNA, 51 bp, synthetic construct
  source 1..51: mol_type = other DNA
gtacaggaaagaactatatttttccaggatgacgggaactacaagacacgt

SEQ ID NO: 70 - DNA, 30 bp, synthetic construct
  source 1..30: mol_type = other DNA
atcctggaaaaatatagttctttcctgtac

SEQ ID NO: 71 - DNA, 51 bp, synthetic construct
  source 1..51: mol_type = other DNA
gtacaggaaagaactatatttttcgatgatgacgggaactacaagacacgt

SEQ ID NO: 72 - DNA, 30 bp, synthetic construct
  source 1..30: mol_type = other DNA
atcatcgaaaaatatagttctttcctgtac

SEQ ID NO: 73 - DNA, 51 bp, synthetic construct
  source 1..51: mol_type = other DNA
gtacaggaaagaactatatttttctgcgatgacgggaactacaagacacgt

SEQ ID NO: 74 - DNA, 30 bp, synthetic construct
  source 1..30: mol_type = other DNA
atcgcagaaaaatatagttctttcctgtac